European Patent Application EP 4 733 386 A1, published April 29, 2026. Title: BIFIDOBACTERIUM ANIMALIS STRAIN, PROBIOTIC PREPARATION, PREPARATION METHOD AND USE THEREOF. Applicant: COREE COMPANY LIMITED. The sequence listing filed with the application follows.

SEQUENCE LISTING (9 sequences)

SEQ ID NO: 1 - DNA, 1400 bp, Bifidobacterium animalis subsp. lactis
  source 1..1400: mol_type = other DNA
  misc_feature 1..1400: note = 16S rRNA gene
tgcagtcgaacgggatccctggcagcttgctgtcggggtgagagtggcgaacgggtgagtaatgcgtgaccaacctgccctgtgcaccggaatagctcctggaaacgggtggtaataccggatgctccgctccatcgcatggtggggtgggaaatgcttttgcggcatgggatggggtcgcgtcctatcagcttgttggcggggtgatggcccaccaaggcgttgacgggtagccggcctgagagggtgaccggccacattgggactgagatacggcccagactcctacgggaggcagcagtggggaatattgcacaatgggcgcaagcctgatgcagcgacgccgcgtgcgggatggaggccttcgggttgtaaaccgcttttgttcaagggcaaggcacggtttcggccgtgttgagtggattgttcgaataagcaccggctaactacgtgccagcagccgcggtaatacgtagggtgcgagcgttatccggatttattgggcgtaaagggctcgtaggcggttcgtcgcgtccggtgtgaaagtccatcgcctaacggtggatctgcgccgggtacgggcgggctggagtgcggtaggggagactggaattcccggtgtaacggtggaatgtgtagatatcgggaagaacaccaatggcgaaggcaggtctctgggccgtcactgacgctgaggagcgaaagcgtggggagcgaacaggattagataccctggtagtccacgccgtaaacggtggatgctggatgtggggccctttccacgggtcccgtgtcggagccaacgcgttaagcatcccgcctggggagtacggccgcaaggctaaaactcaaagaaattgacgggggcccgcacaagcggcggagcatgcggattaattcgatgcaacgcgaagaaccttacctgggcttgacatgtgccggatcgccgtggagacacggtttcccttcggggccggttcacaggtggtgcatggtcgtcgtcagctcgtgtcgtgagatgttgggttaagtcccgcaacgagcgcaaccctcgccgcatgttgccagcgggtgatgccgggaactcatgtgggaccgccggggtcaactcggaggaaggtggggatgacgtcagatcatcatgccccttacgtccagggcttcacgcatgctacaatggccggtacaacgcggtgcgacacggtgacgtggggcggatcgctgaaaaccggtctcagttcggatcgcagtctgcaactcgactgcgtgaaggcggagtcgctagtaatcgcggatcagcaacgccgcggtgaatgcgttcccgggccttgtacacaccgcccgtcaagtcatgaaagtgggtagcacccgaagccggtggcccgacccttgtgggggga

SEQ ID NO: 2 - DNA, 10 bp, synthetic construct
  source 1..10: mol_type = other DNA
  misc_feature 1..10: note = OPA-02 primer
tgccgagctg

SEQ ID NO: 3 - DNA, 10 bp, synthetic construct
  source 1..10: mol_type = other DNA
  misc_feature 1..10: note = OPA-18 primer
aggtgaccgt

SEQ ID NO: 4 - DNA, 10 bp, synthetic construct
  source 1..10: mol_type = other DNA
  misc_feature 1..10: note = OPL-07 primer
aggcgggaac

SEQ ID NO: 5 - DNA, 10 bp, synthetic construct
  source 1..10: mol_type = other DNA
  misc_feature 1..10: note = OPL-16 primer
aggttgcagg

SEQ ID NO: 6 - DNA, 10 bp, synthetic construct
  source 1..10: mol_type = other DNA
  misc_structure 1..10: note = OPM-05 primer
gggaacgtgt

SEQ ID NO: 7 - DNA, 18 bp, synthetic construct
  source 1..18: mol_type = other DNA
  misc_feature 1..18: note = 27F primer
agtttgatcmtggctcag

SEQ ID NO: 8 - DNA, 19 bp, synthetic construct
  source 1..19: mol_type = other DNA
  misc_feature 1..19: note = 1492R primer
ggttaccttgttacgactt

SEQ ID NO: 9 - DNA, 891 bp, Bifidobacterium animalis subsp. lactis
  source 1..891: mol_type = other DNA
  misc_feature 1..821: note = tuf gene
ggtatcaccatcaacattgcccacatcgagtaccagacggccaagcgtcactacgcccacgtcgactgcccgggccacgccgacttcgtgaagaacatgatcaccggcgctgcccagatggatggcgccatcctcgttgtggccgccaccgacggcccgatggcccagacccgcgagcacgtgctgctcgcccgtcaggtcggcgtcccgaagatcctcgtcgctctgaacaagtgcgatatggtcgatgacgaagagctcatcgagctcgtcgaagaagaggtccgcgacctcctcgacgagaacggcttcgaccgcgactgcccggtcgtgcacacctccgcttacggcgctctgcatgacgacgctccggatcacgacaagtgggttgccaccatcaaggagctcatggacgacgtcgacgagtacatcccgaccccggtccacgacctcgacaagccgttcctgatgccgatcgaggacgtcttcaccatctccggccgtggcaccgtcgtcaccggtcgtgtcgagcgcggcaagctgccgatcaacacgaacgtcgagatcgtcggcatccgcccgacccagaccaccaccgtcacctccatcgagaccttccacaagcagatggatgagtgcgaggccggcgacaacaccggtctgctgctccgcggcatcaaccgcaccgacgtcgagcgtggccaggtcgtggctgctccgggttcggtcaccccgcacaccaagttcgaaggcgaagtctacgtccttaccaaggatgagggcggccgtcactcgccgttcttctcgaactaccgtccgcagttctacttccgcaccaccgacgtcaccggcgtcatcacgctgccggaaggcgtcgagatggttcagcct